European Patent Specification EP 4 051 700 B1, published May 7, 2025. Title: NUCLEIC ACIDS ENCODING ANCHOR MODIFIED ANTIBODIES AND USES THEREOF. Applicant: Regeneron Pharmaceuticals, Inc. Mastaitis, Jason Murphy, Andrew J. McWhirter, John Voronina, Vera Gromada, Jesper. The sequence listing filed with the application follows.

SEQUENCE LISTING (32 sequences)

SEQ ID NO: 1 - DNA, 855 bp, Homo sapiens
gagacagggacagacgtaggccaagagaggggaaccagagaggaaccagaggggagagacagagcagcaagcagtggattgctccttgacgacgccagcatgagctccttctccaccaccaccgtgagcttcctccttttactggcattccagctcctaggtcagaccagagctaatcccatgtacaatgccgtgtccaacgcagacctgatggatttcaagaatttgctggaccatttggaagaaaagatgcctttagaagatgaggtcgtgcccccacaagtgctcagtgagccgaatgaagaagcgggggctgctctcagccccctccctgaggtgcctccctggaccggggaagtcagcccagcccagagagatggaggtgccctcgggcggggcccctgggactcctctgatcgatctgccctcctaaaaagcaagctgagggcgctgctcactgcccctcggagcctgcggagatccagctgcttcgggggcaggatggacaggattggagcccagagcggactgggctgtaacagcttccggtactgaagataacagccagggaggacaagcagggctgggcctagggacagactgcaagaggctcctgtcccctggggtctctgctgcatttgtgtcatcttgttgccatggagttgtgatcatcccatctaagctgcagcttcctgtcaacacttctcacatcttatgctaactgtagataaagtggtttgatggtgacttcctcgcctctcccaccccatgcattaaattttaaggtagaacctcacctgttactgaaagtggtttgaaagtgaataaacttcagcaccatggacagaagacaaa

SEQ ID NO: 2 - protein, 151 aa, Homo sapiens
MSSFSTTTVSFLLLLAFQLLGQTRANPMYNAVSNADLMDFKNLLDHLEEKMPLEDEVVPPQVLSEPNEEAGAALSPLPEVPPWTGEVSPAQRDGGALGRGPWDSSDRSALLKSKLRALLTAPRSLRRSSCFGGRMDRIGAQSGLGCNSFRY

SEQ ID NO: 3 - protein, 5 aa, Homo sapiens
NSFRY

SEQ ID NO: 4 - DNA, 15 bp, Artificial Sequence
  G4S DNA sequence
  CDS (1)..(15)
ggtggcggcggtagc

SEQ ID NO: 5 - protein, 5 aa, Artificial Sequence
  Synthetic Construct
GGGGS

SEQ ID NO: 6 - DNA, 107 bp, Homo sapiens
gcagctacaggtaaggggcttcctagtcctaaggctgaggaagggatcctggtttagttaaagaggattttattcacccctgtgtcctgtccacaggtgtccagtcc

SEQ ID NO: 7 - protein, 19 aa, Homo sapiens
MDWTWRFLFVVAAATGVQS

SEQ ID NO: 8 - DNA, 327 bp, Artificial Sequence
  ANP-VH1-69 without leader
  CDS (1)..(327)
aacagcttccggtacggtggcggcggtagccaggtccagctggtgcagtctggggctgaggtgaagaagcctgggtcctcggtgaaggtctcctgcaaggcttctggaggcaccttcagcagctatgctatcagctgggtgcgacaggcccctggacaagggcttgagtggatgggagggatcatccctatctttggtacagcaaactacgcacagaagttccagggcagagtcacgattaccacggacgaatccacgagcacagcctacatggagctgagcagcctgagatctgaggacacggccgtgtattactgtgcgagagac

SEQ ID NO: 9 - protein, 109 aa, Artificial Sequence
  Synthetic Construct
NSFRYGGGGSQVQLVQSGAEVKKPGSSVKVSCKASGGTFSSYAISWVRQAPGQGLEWMGGIIPIFGTANYAQKFQGRVTITTDESTSTAYMELSSLRSEDTAVYYCARD

SEQ ID NO: 10 - DNA, 583 bp, Artificial Sequence
  ANP-VH1-69 Cas9/BHR donor
ctcgagcagctacaggtaaggggcttcctagtcctaaggctgaggaagggatcctggtttagttaaagaggattttattcacccctgtgtcctgtccacaggtgtccagtccaacagcttccggtacggtggcggcggtagccaggtccagctggtgcagtctggggctgaggtgaagaagcctgggtcctcggtgaaggtctcctgcaaggcttctggaggcaccttcagcagctatgctatcagctgggtgcgacaggcccctggacaagggcttgagtggatgggagggatcatccctatctttggtacagcaaactacgcacagaagttccagggcagagtcacgattaccacggacgaatccacgagcacagcctacatggagctgagcagcctgagatctgaggacacggccgtgtattactgtgcgagagacacagtgtgaaaacccacatcctgagagtgacaaaaaccctgagggcgccggcggaattcaagcttcctaggcgccggcgagaaggcagctgtgccgggctgaggagatgacaggggttattaggtttaaggctgtttactcgag

SEQ ID NO: 11 - DNA, 19726 bp, Mus musculus
aagcttatctctctgttgctcagactcatctaggaatttcagaaatttctgttctagcatctcttccagcttttgtctccaaccctcattctcttctttctttttttttttaaattatatgttctctgtctttttaaaaaactttttaaaattaggtatttatgtcatttacatttccaatgctatcccaaaagtcccacccacgctccccaacccactatcccacccacccactcccacttcttggccctggcattcacagtgtactgagacatataaagtttgcacaaccaatgggcctctctttccactgatggccgactaggccatcttctgatacatatgcagctagagacacgagattctgggggtactggttagttcatattgttgttccacctatagggttgcagatccttttagctccttgggtactttctctagctcctccattgggggccctgtgatccatccaatagctgactgtgagcatccacttctgtgtttgctaggccccagatagtctcacaagagacagctatatctgggtcctttcagcaaaatcttgctagtgtatgcaacggtgtcagagtttggaagctgattatgggatggatccccggatatggcattctctagttggttcatccttttgtctcagctccaaactttgtctctgtaactccttccatgggtgttttgttcccagttctaaggaggggcaaagtatccacactttggtcttcattcttcttgagtttcatgtgttttgcaaattgtatcttatatcttgggtattctaagtttctgggctaatatccacttatcagtgagtacacattgtgtgagttcttttgtgattgggttacctcactcagtatgatgccctccaggtccatccatttgcctaggaatttcataaattcattctttttaatagctcagtagtactccattgtgtagatgtaccacattttctgtattcattcctctgttgaggggcatctgggttctttccagcttctggctattataaataaggctgctatgaacatagtggagcatgtgaccttcttaccggttgggacatcttctggatatatgcccaggagaggtattgctggatcttccggtagtactatgtccaattttctgaggaactgacaaactgatttccagagtggttagtaccagcttgcaatcccaccaacaatgagaggagtgttcgtctttctccacatcctcaccagcatgctgctgtcacctgaatttttgatgcttagccattctgactggtgtgaggtggaatctcagggttgttttgatttgtatttccctgatgattaaggatgctgaacattttctcaggtgcttctcagccattcagtattctttaggtgagaattctttgtttagctctaagccccatttttttaatggggttatttgattttctggagtccaccttcttgagtttttttttccattttttattacataatttcctcaattacatttccaatgctatcccaaaagtcccccataccctcccccccccaattccctacccaccccttcccatttttttggccctggcgttcccctgtactggggcatataaagtttgtgtgtccaatgggcttctctttccagtgatggctgactaggccatcttttgatacatatgcagctagagtcaagagctcccgggtactggttagttcataatgttgttccacctatagggttgcagatccctttagcttcttgggtactttctctagctcctccattgggagccctgtgatccatccaatagctgactgtgagcatccacttctgtgtttgctaggccccggcatagtctcacaagagacagctacatctgggtccttttgataaaatcttgctagtgtatgcaagggtgtcagcatttggaagctgattatggggtggatccctggatatggcagtctctacatggtccatccttttgtctcagctccaaactttgtctctgtaacttcttccatgagtgttttgttcccaattctaaggaggggcatagtgtccacacttcattcttcattcttcttgagtttcatgtgtttagcaaattgtatcttatatcttgggtatcctaggttttgggctaatatccacttatcagtgagtacatattgtgtgagttcctttgtaaatgtgttacctcactcaggatgacgccctccaggtccatccatttggctaggaatttcataaattcattctttttaatagctgagtagtactccattgtgtaaatgtaccacattttctgtactcattcctctgttgaggggcatctgggttctttataggttctggctattataaataaggttgctatgaacatagtggagcatgtgtccttcttaccggttgagacatcttctggatatatgcccaggcgaggtattgctggatcctccggtagtactatgtccaattttctgaggaactgccagactgatttccagagtggttgtacaagcctgcactctcaccaacaatggaggagtgttcctctttctccacatccacgccagcatctgctgtcacctgaatttttgatcttagccattctgactggtgtgaggtggaatctcagggttgttttgatttgcatttccctgatgattaaggatgttgaacatttttttcaggtgcttctctgccattcggtattcctcaggtgagaattctttgttcagttctgagccccattttttaatggggttatttgattttctgaagtccaccttcttgagttctttatatatgttggatattagtcccctatctgatttacgataggtaaagatcctttcccaatctgttggtggtctttttctcttattgacggtgtcttttgccttgcagaaactttggagtgagttctttatatatattggatattagtcccctatctgatttaggataggtaaagatcctttcccaatctgttggtgacctttttgtcttattgacggtgtcttttgccttgcagaatctttgcaattttatgaggtcgcatttgtcaattctcgatcttacagcacaagtcattgctgttctgttcaggaatttttcctctgtgcccatatcttcgaggcttttacctgctttctcctctatatgtttgagtgtctctggtttaatgtggagttccttaatccacttagatttgaccttagtacaaggagataggaatggatcaattcgcattcttctacatgataaccgctagttgtgccagcaccatttgttgataatgctgtcttttttccactggatggtttttgctcccttgtctaagatcaagtgaccataggtgtgtgggttcatttctgggtcttcaattctatttcattggtctacttgtctgttgttataccagtaccatgcagattttatcacaattgctctgtagtagagttttaggtcaggcatggtgattacaccagaggttttttttatccttgagcagagtttttgctatcctaggttttgtgttatttcagatgaatttgcagattgccctttccagttcgttgaagaattgagttggaattttgatggggattgcattgaatctgtagattgctttggcaatatagccatttttactatattgatcctgccaatccatgagcatgggagatctttccatcttctcaaatcttctttaatttctttcttcagagacttgaagttcttgtcatacagatctttcacttccttagttagagtcacgctaaggtattttatattatttgtgactattgagaagggtgttgtttccctaatttctttctcagcctgtttatcctttgtgtacagaaaagccattgacttgtgttagttaatctcatatccagctacttcactgaagcggtttatcaggtttaggagttctctggtgtaatttttagggtcactcatatatactatcatatcatctgcaaaaagtgacattttgacttcttcctttccaatttgtatccccttgatctccttttgttgtcgaattgctctggcaaggacatcaagtactatattgaataggtagggagaaaatcggcacccttgtctagtccctgattttagtaggattgcttcaagtttctcaccatttactttgatgttggctactggtttgctgttgaatgctttttatcatgtttaggtatgggccttgaattcctgatctttccaagacttttatcatgaaagggtgttggattttgtcaaatgctttctccagcctttcattctgaggttgtgtctgtctttttccctgagatgggtttcctgtaagcagcaaaatgttgggtcctgtttgtgtagcccgtctgttattctatgtctttttattggggagttgagtccattgatattaagatatattaaggaaaagtaattgttgcttcctattatttttgtttttaaagttggcattctgttcttgtggctgtcttcttttaggtttgttgaaggattcctttcttgctttttctaggtcgtggtttccatccttgtattcattttttttctgttattatcctttgaaggactggattcatggatagataatgtgtgaatttggttttgtcttggaatacttttgtttctccatctacggtaattgagagtttggctgggtatagtagcctgggctggcaattgtgttgtcttagtgtctatataatgtctgtccaggatcttctggctttcatagtctgtggtgaaaaatctggtgtaattctgataggcttgcctttatatgttacttgaatttttcacttactgcttttaatattctttctttatttagtgcatttgttgttctgattattatgtgtcgggaggaatttcttttctggtccagtctatttggagttctgtaggcttcttgtatgttcacgggcatctctttctttaggtttgggaagttttcttctataattttgttgaagatatttgctggcccttcaagttgaaaatgttcattctcatctactcctattattcgtatggttggtcttctcattgtgtcctggatttcctggatgttttgagttaggatctttttgcattttccattttctttgattgttgtgcagatgttctctatggaatcttctgcacctgatattctctcttccatctcttgtagtctgttgctgatgctcgcatctatggttccagatttctttcctagggtttctatctccagtgttgccccactttgggttttctgtatagtgtctacttccctttttagatctagtatggttttgttcatttccatcacctgtttgggtgtgttttcctgtttttctttaaagacttgcaactctttagcagagttctcctgtatttaagtgagttattaaagtccttcttgatgtccagtaccataattgtgagatatgcctttaaatccaagtctaggtttttgggtgtgttggggtgccctggactggctgagttgggagtgctgcattctgatgatggtgagtggtcttggtttctgctagtaagattcttacatctgcctttcgccatctggtaatctctggagtcagttgttaaagttgtctctggttaaagcttgttcctctcgtgattctgttattctcttccagcagacctgggagactagctctttcctgagtttcagtggtcagagcactctctgcaggcaggatttcctctttcagggaaggtgcacagatatctggtgttcagatttgcctcctggcagaagatgatggcctgaaacaggacctgtcccagaagctgttagcttctgtagtcaacactgtcacctgtgcagactagtctcggtggagtccgggaaccaagatgtctcctgcagatgctctggcattcccttctgggccgggtgatcacctctcctctggcagggaaggtgccctggtgtctggaacccgaaaagggggctgcctcagaagctctgtggctactgcctgtcccagaagctgttagcttctgtagtccacactctcacctgtgcagactagtcttggtggagtctgggaaccaagatgtctcccgcagatgctccagccattctcctctttctgttgcttattttgacctatgaaatcctggacatatagttctagtgttgcttgtaatctcttttctaagccaaggaattttttttatctagggcacaatcttttgagaagacatattaaatcaagagaataaatattgcaagaccaataaatgataaggtatctattttctttaaatccatcgctgtcaaaccattcaaaatatcctcacataaagccaaaaagatatttattgtgtttcccatcttagttgagttcaagtcaatattttggtgccattttgttgcagtaaatctctaacacaaatatgcctgggcaatgaaaacacaactcagttaatatgaatacagattgttcagatctaccactacactaccatcttcttcatctaagagaccccttagaacttgcagtttctccaggccttgtgcttctgcgctgcttttcttcttcttcctcttctacattgcttctctcataaacctacttctttttttccctccttctgttccatcttcccttttatctgcccaatcattagctctcctttattttacaaattaaggtgtgaagccggtttctaggaaatcacctgagtgctgacttgttccttgttcagagccacgcacaggagaacagaattaacatcaaatataattatccccagggctatccacaacacgtgcatcctataagatcaccacggactaatgctggtcttcaattacaacataaacaacaaaaaccccacatatatgtggaaacaaatcgaactatacaaagaatcaatgaaaccaggagcttgttctttgagaaaaatcaacaagatagataaacccttagccagactaaccagagggcacagagacagtatccaaattaataaagtcagaaatgaaaggaagacataacaatgaaatatatcttaaaataattaatctgtttgtagactattagcagttgaaaatattaaaatcatgttctacaaacgtggaattattattgataattttctcactgtgcttgaaattagcattttcttaatgtttaacttcaaagagtttttgctattttgaaatattaaacatatacttactgataaaataatttccctcctaacaacactgataatctttttttaagtaaactgattattagacaatgtacacagatatataatgtgttttaaatactctcccactgtcaggtggtatcatatagggcctttgaatatatttttaaatgtattatttgtaatattttatggtctctcctatgcttatttctgaaagaatattttgtatgttttgaaacaatttagtatttaacattagatataggatcctcagttatggatagtattaaatattcattaatgatatttttaaggtataaaaggatatgaatataaaagtttaacaaattttatgtattatttgattctaaaaatactcaatattattaatatgtttgatgtttaaaatgcatttaaataataaaaacatttaaaaaaataaaatcaagaaatgaggttctaagcagaggtcaaggaaaatgaggaatagaaaaatagtaaaaatcaatatgtccatttattcaaggaaagctcctacatagacattgcaccagattagcaaatattatggtcctcatattagtttaagttaggagactatgcttatgttatctatttacattctaaggagcctagacatttgtgaatggattacattataagaggaggatgtctacttaagtaggcatgaacgcctgtgcattgcaccctatgagttccatcagcattccatgattggagtatgaagaacagcattatagacattacccagaaccttagtggttctagaatgccaagataaaacaatctaaccttctggatagtagggataaatgttcctatatcatcagaattcactggtgccctgaggatgttaccctgctaactgacaattcacaggacatcacatggattctgataagttgcagaaaagaggagatgcattcaattggtcctcctccttctaagctgcaatattaggtgcatccaatttgtgaacttcaatttagattacaatagacatgaataatctgaattcatgtagtacatatttttgttttaatatgagttaccattgttcagaaaattaaatacacatgatcacatattcctacatagtgctgttagtttttcacatctctgggacaatattccaaatatctccttcattagtgaaaatatcaactactgtaaagcttagctaacatgcctttgcaggaataagaacatcctggattgaaagctacacagggagatgtaaaactttctaagcacacacattctccatccattaggatcatggtccatgagatttttctctctctcttcttcccattaaatgcatgtacatgcaggttgggaaacagattgtgttgcagaatacatttgcttgatttccacttccttctcaatgcaaatatttttgaagtgttaattttgctgtgagtaccacagtggttcttgctctttctgttgactcctgtctgtgaatgttccaggaattcacacatggacacacgtggggctgcatctgagctccagactcactgttgtccttctgtcctcagctgctctggcccaggcacagcctcgtgaattcaacaaagaccctgatctctcttgtttacacctcattacaaatgggaactgttagaggtggacccaactgcatttccatgaggaaagcacatgagtttgagagggtcgttgatgataaggtagaaacaactttaattcataggctgagatatcagtcatcacctccagataaacaagagccatttcttcctgcatctgagccctgtaagcacactagctttaggaatatgttactgctgaagtcagattgggcaacttcatagtatacaatagaaaatctacctgcagatgagttcagaaccagcagggggcacaatggggccaagaatccctagcagagagatgtggtgtgtgtgcaggggactctgcatcctctgtggtttcctttcttaacttacatgtacctgtagtgattgacatgtaacgtttccacgctcaaacactgtgaagatactttgctaaacacttcaaagatttatgttttcttgatgtgtgcatgtgtgtattcttttttgtttttagacacagggtttctctgtgtagtcctggctgccctggaactcactctgtagaccaggctggcctcgaactcagaaatctgcctgcttctgcctcccaagtgctgaagttaaagacatgtgccaccattgcctggccatgtgtgtattcttgatgcactcttctgttgacagatacacagtttatttccataatttatttattgtgatggtgctgcaataatcacttatgtacaaatgtttctgaagtatatttagttttggtcatttgggtgattatttttttctttctagtatatagcattttggaaaggtagatattaattgtatgtatgggaaggaggctgtaaattctaataacttagctgcttttgaaatttgtcctcaattctatcatccttgtaaccaccttaaatccatctattagccttgtcacaagtgagccactgtctcaggctgcaaatctttttatagattaggtcgtgatgttacatccacagcctctgcacaatgctcaggggtgggatatgggatgaattccctcagacagcattaggacttggatctcagcagactgattcttgacccaaatgtctcttcttctctagcaggagtaagtccttatctaagatgtactctgctcatgaatatgcaaatcaattgagtctatggtggtaaatatagggatgtctacacccctcaaaaacttaagatcactgtcgtcttcacagtcacaggagtacacaggacatcaccatgtgttggagctgtatcatcctcttcctgttagcaacagctgcacgtaaggggcttacagtagcaggcttgaggtctggccatacactcatgtgacaatgacatccactctgtccttcccttcacaggtgtgcactcccaggtccagctgcagcagtctggggctgagctggtgaggcctggggcctcagtgaagatttcctgcaaggcttttggctacaccttcacaaaccatcatataaactgggtgaagcagaggcctggacagggcctggactggattggatatattaatccttataatgattatactagctacagaaccagaagttcaagggcaaggccacattgactgtagacaaatcctccagcacagcctatatggagcttagcagcctgacatctgaggactctgcagtctattactgtgcaagacacagtgctacaaacacatcctgagtgtgtcagaaaccctggaggagaagcaagcagagctggaatggagatgacagaaagattatcatttagacttgctcagaaagagaaattttgaatgcccatttattgcctcttccttacagtactatagtgcctgtttttgttgacattttcaaactaatttccaaagtcactaccacaatttacaatcacataaaaagcaagcaaggataacattattttctgtgcttacttgccatttatattcttgcttattctcatctcactgaggtcatattgggacattaaatttctggggttactttttattaaaaatttttcattattcattcactttacatccttctagtcttcctctcacacatgccctatccctttctcctctgagaggatggagccctccctaccctcgtatccccttacccaggcacatcaagtgtctgcagtactaggaatattctctgtcaatgctgccagacaaggcagacaagttaggggatcaggattcacaggaaggcaacagcttgagggacagcccccactgaagttattggtggattcacatgaagactgagttgcacatctgctacatatattcaggggtcctatttacagctcaagtagactcttgttggtggtttagtctcttagaaccccaagtgtccaggttagttgactctgtgggtcttcctttggagttcctatcccctccagatccctcagttcttctcccaactcttccataagacacccgtaggtccatccaatgtttggttttgggtttttctgcatctgcttcagtcagctgctgggtggagcatctctgaggataattatgagaagctcttatgtgcaagcataacaggatatcattattagtgtcagggactggtgcttggccatgggatgggtctcaagtttggtcagttatttggccattcccacagtctctgataatctttgtccctgcatttcttgtagacaggaaaaatattgggttgaaagttttgtgggtgggttggcgtctctattgctccactgggcttctttctggatataggagtttgcctcttcaggttccatattcccaaagtagtgtgtcacactaaggtcactcccatacagagggacactcattctcttgccacgtctctgtccaccttcattggacctgaggttcctgaatcatacagaactgcatgtgtgcaaccacacagaacaaggctatctatcagaggcctaccataccaggaccatcaaggttcaccttactcccaatactgactacaaaaagaacatcaaggaccaatgcagtctatatggataaacacacttgaaagaacacaaacaagattgagggcaacatgacacctccaaagcatacctaaccgagtacagcatgccctggatatcctaacacaatcaaaacacaagaaagttaccttaaatccagtcttataaaggtgatgaaggcctttaaataggaaatgaattaatccttaggataatacaggacaatacattcgaacagatagaggtctttaggaggaaagaaataaatccctcaaagacatacatgaaaatacaattaaacaggtgaaagtaataactacaatggtgtaagacctaaaaatggaaatagaagcaataaagtaacacaaacttagaatcttgaaggtggaaaacctagagaacaggaatactagatgcaaggatgatatcttctaggtccatccatttgcttgcacaatttatcatgtccttgcttttaatagttgaacagtatttcattgtttaaatgaaccacatgttctgtctccattctctggatgagggggtgagcaagtttttccacattctggctattacaaatagagctgctatgaacctagtagaaaacatatcctgtgtatggtggagagttttggagtatatcaccaagagtgttatagctgggtcttcatgtagaactattcctaattttctgagaaatcccaagtcagatttctagaatggttgttcaagtgttcactccaaccatcaatggaggactgttttccttgccagcatgtgctgtattttgagtttttgatcctagccagttttatcctgcatttcacacttagatatggactatggtacaggacagagagaaaccaaccttctactcaccaggatattctacctgctaccaatttatttatttatttatttatttatttatttatttatttatttatttatattagagaacaacaccatgcagtttagaagaagtactaagacgtcagtgatgttatactgtgcctaaccttgcattgtacaatctcagctttcaggtaagacagtgcatgactcttatgcagtgccaactgttttctgattgtatttatggtctattgcctaggaatgacctcctctcaaataaacatggtcaaaagcccatggcctgagatgacagagcccctagtagaccctagttgtatttctgaagtttagatatcataatgacttataaatacttatgtttatacaatagattagagctgctctcagccatgaccaaggagcttctgtgttcaatgaataatgattgatgcagacattcgtgagtggtcaaagtggtgagaatgattagagagtcctcagccacacaagcgttaatgatatgaactttccaatatattaactgtattaatgaataaatgcagacatcatatgagatctcattagtagttcttaggtattgcatttttatatacaattatgcatatcagtacattatagtgtataaaggaaattgtctagcataatagagaaaaataggacagtcaagaaacaaaagagtagaaattatgggtgaaatatgcagtgtgaaatatttacatgaaaattttaaccatatgtaaaattgttatttttgtttttcagaatgagtttgctcattctttgacatttttattcctgtgtgaaatatatcaggatcatatgtatcccattctgatggtctgacttccactgggaatttccaatatatctcttccaactaactgaccagtttctttttttcttattttctctctttctcgttttgttttgctttgttttgtttttcaagacagggtttctctgtgtagctctggctgtcctggaactcactttgtagatcaggctggcttcgagctcataaatccacttgcctctgcctcctgagtgctgggattaaaggagtggctaccacgcccggctagtttttttttttcttataagaacaacatttactggatggtcacttacatattcagaggttcagtcaattattatcaaggcagaagcatggcagtggtccagtagtcatggcactggggaaggagctgagagatctacatcttgctccaaagggaaagaggaatagtctgacttccatgtgtttcagaggagggtttcatttcccacccccacagtgacacacttcctccaacacggccacacctcctaatattgccactcttggatcaagcatattcacaccacaaaggaaagtttagagataaacattaagaaaattaatgaagtcattttatcttatatgctcaacatgactagtacttaaaaccataattttacatgtacaatatttcatggcataacatattttttatatttttattagatattttctttatttatatttcaaatgtgataccctttcccaattcccctccaaaaatcccctatgccttcccctcatagccagctcccaaacccacccactcctgctttctggtcctggcattcccctatactggggcataaaaccttcacaggaccaagtgcctcttctccattgatggccaattaggccatcctctgctacatatgcagctagagccatgagttccaccatgtgttttctttgattggtggtttagttccagggagctctgggggtattggttagttcatattgttcctcctatggggctgcaaaccctttcagccccttgggtattttttctagctccttcattggggaccctgtgctccatccaatggatgagtgagcctccacttttgtatttgtcaggaactggcagagtctctcaggagacaattatatcaggctcctgtcagcaaaatctcgttggcatctgcaatagtgtctgggtttggtggttgtttatgggatggatttctgggtggggcagtctctggattgtcattcctttagtctctgcttccacctttgtctttgtaactccatccatgggtattttgttcccccttcaaagaaggatcaaaatatccacactttagtcttccttcttcttgagtctcatgtgtttttcaaattgtatcttgggtattctgagcttctaggctaatatccacttatcagtgagtgattatcatgtctgttcttttgtgattgagttacctcacttagcatgatatcctccaggtctatccatttgtctaagaatttcataaagtcattgtctttaatagctgcatcgtactcaattgtgtaaatgcaccacattttctttatccattcctctgttgagggacacttggtttttcccagcttctggttattataaataaggctgctatgaacatagtggaacatgtgtccttagtacatgttggaacatcttctgggtatatgcccaggagtggtattgctggatcttctggtggtactatgtccaaatttttggggaaccatcaaactgatttcctgagtggttgtacaagcttgcaatcccacaccagcaatagtggaatgttcatctttgtccaagtccttgccagcatctgctgtcacctgagtttttgatcttagccattcttactggtgtgaggtggaatcttggggttgttttgatttgcatttccctgatgtttaagggttttgaacatttttaggtgcttattagacatttggtattcctcagtttagaaatctttgtttagctctgtaccacatttttgaatagggttatttggttttctggagtctaacttcttgagttctttgtacatattggatattagccctctatcagatttagaattagtaaggatctttccccaaactgttggtggttcttttgtcttattgacagtgtactttgccttagagaagctttgcaattttatgaggtcccatttgtcaattcttgatcttatagtacaagccattggtcttttgttcaggaatttttcccatgtgtccatatgttcaaggcatttccccactttctccactacaagttttagtgtctctggttttatgtggaggtccttgatccacttagatttgagctttgtacaaggagataagaatggatagattcacattcttctacatgctctctgccagttgagctagcaccatttgttgaaaatgctgtcttttttttcccccactggatggtttttagctcttttggccaagatcaagtgaccattggtgtgtgggttcatttcttggtcttcaattctagttcactgacttacctgtttgtcactgtacaaggaccatgcagcttttttcacaattgctctgtagtacagcttgaggtctgggatggtgattctaccagagagattcttttactgttgtgaataatttttgctatcataggatatttttttatttcagatgaatttacaaattgctctttctaactctgtgaacaattgagttggaattttgattgtgattgctttgaatactcaagatataatttacaaaacacatgaaacttaacaaggactactaaagtgcagatacttcgatccttcttagaagggggaacaaaatacccatagatggagttacagagacaaagttcggagcagagactataggaacgaccatccagaggtccacctggggatccatcatgtaaacaaccacccaaaacagacactattgtggatgccaagaagaacttgctgacaggagtctgatatagctgtctcttgagaggctctgccagggcctcagaaagtggaggctcacagccatccattggatggagcacagggtccccaatgaaggagctagagaaagtactcaaggagctgaaggggtttgcagccccataggaggaacaacaatatgaactaaccagtacccccagagctccctgggactaaaccaccaatcaaagaaaacacatggagggacttgaagctcttgctgcatttatagcagaggatggcctagatggtcatcaatgggaggagaggtcaatggtcctgggaaggttccatgccccagtataggggaatgccagggccaggaagcaggagtgggtgggctggggatcagggagggggagatgatagggcattttcagtggggaaactaggaaagaggataacatttaaaatataaataaagaaaatatctaattaaaaaggattacctatgtgcatgggagctcatgagcagcaggggtcactctaaggccaataatccacatagagcgatgagctgtgtgtgaacaggactctgtatcctctgtggtttcctttcttaagtgtattaactgatctgtccagctgtgattgacatgtgatgtctccatgctcaagcccagtaaagattctctgttaaataccttacagacttatgtttacttgtttttatttgcttttcatatttttttaaaaagtcatacaatgtattctaataactcattctcccatctccaatttattctaagtttttcttaactcatccaaccacacactttttaattctgataaagcacccccccccccaaaaaaaaacccaaccaaccaaaaaaaaaaaaagccaaggaatttaaaaggggattgaaagcaaataaaaactaaacaaaaaagtaaaaactacacacacacacacacacacacacacacacacacacacacacacacactcacacacacacacacacaccacacacacacacacccatgcacgaacacacacacacacacacacacacacacacacacacacacacacacacacacatggaatccagtaaaaccacaactctttacccatgatacacaggaaaatataagtcaaacaaacagaatggaagaaggtggtattataaaaatgtctgcacaaataccattaagttcattttcttgttggctaccaactgctaagcctgtctcccttgattaattgtgcttatcatcccctatgaactccattggaggacactaatttttccttctgtctccaggaattgaagtgttgcagaactctcagtagctttatttacctgcacaatacagcctctaatccaaccagtgaaaattaccacatgagagacttccaaatgaaagaacaggtaaagttgtctactggcaagcttagtaatatcatgtaaatgccttagaatttaatgacatatgtcatcctctgaggttaataaatccattttggtgcatatataccctgaactcaccactaacataatacaacaattaaaaaattccaacatggatgcagaggaatccctgagggacatttgttgatttgtgagcacaatataattattttttgggggggaaatgtctgaatgttaactctttaccagtgataatctattctattaatgtgtacataggtagcactaattaaaatcactgtgttatcaggtaatgaaacagaggaagtaggatgctgggaaacagacttttggaaggtcccaagggaaaccacagggacctagtggtgatagattatggtgagagtcctgagagtggtcatagattatagcatatttcatatgcaattgaaaatttcaaagaatgaaaatccttatgaaatatagaaataacaactttacttatgtacatatacttcatagtacaatttttacactgtgcatatttctcctgtaacatctggttcctcctattttcctttattctcctagacaatttcactgatacaatctcatgtttttgtataaatagttgtatataactattaaatacataagctgttaatgagtcttcattaatgtctgtgatttttttattgtcttaattaatactattatctctaattgcatccacattttcaaaagcaatgtaaatttcttactcatttctgttcaaaaacttctgttgttgtatcattaccatgccttagtgataaaatcctttcttgacacatctatagctattgctataatttagttattgatgatcctcctgcaataatcattgataggtaaatattttaagcacttttacttttagtcattttagtgagatttgaagtagtatataacctgttggaaaggcaaatattaattccatatatgtgaaagaagacgctaaaactaaaaacattagccacttttagatatcttctccttcttcttcttcttcttcttcttcttcttcttcttcttcttcttcttcttcttcttcttcttcttcttcttcttttcttcttcttcttctccttctccttctccttctccttctccttctcctcttcctcctccttccttccttccttccttccttccttccttccttccttccttccttccttccttccttccttccttccttccttccttccttccttccttccttccttccttccttcctttctttctttctttctttctttctttctttctttctttctttctttctttctttctttctttctttctttctttctttctttcttctcctcctccttctttttccttctccttccccttcaccttccccttccttcctctttcccttccccttctccttctcctcaatctacaatctgttaacatattaacatgtcccagagtagagcaacagactcaggtcaaacatctactgagaaatttgcccatgtagttaacatctacagcatctgtctaggggttacaaaaagtctatgggatacaattcctcagaaaggaataggatttggacctgagcatactgctgcctaacacatgaaatggcagttcttctccagctggactaggtccttaactaagaaatgcactgctcatgaatatgcaaattacccaagtctatggcagtaaatacagagatgtccacaccctgaagacaacctatgaacaatgttctctccacagtccctgaagacactgattcta

SEQ ID NO: 12 - DNA, 7928 bp, Mus musculus
ctgagcattgcagactaatcttggatatttgtccctgagggagccggctgagagaagttgggaaataaactgtctagggatctcagagcctttaggacagattatctccacatctttgaaaaactaagaatctgtgtgatggtgttggtggagtccctggatgatgggatagggactttggaggctcatttgagggagatgctaaaacaatcctatggctggagggatagttggggctgtagttggagattttcagtttttagaataaaagtattagctgcggaatatacttcaggaccacctctgtgacagcatttatacagtatccgatgcatagggacaaagagtggagtggggcactttctttagatttgtgaggaatgttccacactagattgtttaaaacttcatttgttggaaggagagctgtcttagtgattgagtcaagggagaaaggcatctagcctcggtctcaaaagggtagttgctgtctagagaggtctggtggagcctgcaaaagtccagctttcaaaggaacacagaagtatgtgtatggaatattagaagatgttgcttttactcttaagttggttcctaggaaaaatagttaaatactgtgactttaaaatgtgagagggttttcaagtactcatttttttaaatgtccaaaattcttgtcaatcagtttgaggtcttgtttgtgtagaactgatattacttaaagtttaaccgaggaatgggagtgaggctctctcataacctattcagaactgacttttaacaataataaattaagtttcaaatatttttaaatgaattgagcaatgttgagttggagtcaagatggccgatcagaaccagaacacctgcagcagctggcaggaagcaggtcatgtggcaaggctatttggggaagggaaaataaaaccactaggtaaacttgtagctgtggtttgaagaagtggttttgaaacactctgtccagccccaccaaaccgaaagtccaggctgagcaaaacaccacctgggtaatttgcatttctaaaataagttgaggattcagccgaaactggagaggtcctcttttaacttattgagttcaaccttttaattttagcttgagtagttctagtttccccaaacttaagtttatcgacttctaaaatgtatttagaattcattttcaaaattaggttatgtaagaaattgaaggactttagtgtctttaatttctaatatatttagaaaacttcttaaaattactctattattcttccctctgattattggtctccattcaattcttttccaatacccgaagcatttacagtgactttgttcatgatcttttttagttgtttgttttgccttactattaagactttgacattctggtcaaaacggcttcacaaatctttttcaagaccactttctgagtattcattttaggagaaagactttttttttaaatgaatgcaattatctagacttatttcagttgaacatgctggttggtggttgagaggacactcagtcagtcagtgacgtgaagggcttctaagccagtccacatgctctgtgtgaactccctctggccctgcttattgttgaatgggccaaaggtctgagaccaggctgctgctgggtaggcctggactttgggtctcccacccagacctgggaatgtatggttgtggcttctgccacccatccacctggctgctcatggaccagccagcctcggtggctttgaaggaacaattccacacaaagactctggacctctccgaaaccaggcaccgcaaatggtaagccagaggcagccacagctgtggctgctgctcttaaagcttgtaaactgtttctgcttaagagggactgagtcttcagtcattgctttagggggagaaagagacatttgtgtgtcttttgagtaccgttgtctgggtcactcacatttaactttccttgaaaaactagtaaaagaaaaatgttgcctgttaaccaataatcatagagctcatggtactttgaggaaatcttagaaagcgtgtatacaattgtctggaattatttcagttaagtgtattagttgaggtactgatgctgtctctacttcagttatacatgtgggtttgaattttgaatctattctggctcttcttaagcagaaaatttagataaaatggatacctcagtggtttttaatggtgggtttaatatagaaggaatttaaattggaagctaatttagaatcagtaaggagggacccaggctaagaaggcaatcctgggattctggaagaaaagatgtttttagtttttatagaaaacactactacattcttgatctacaactcaatgtggtttaatgaatttgaagttgccagtaaatgtacttcctggttgttaaagaatggtatcaaaggacagtgcttagatccgaggtgagtgtgagaggacaggggctggggtatggatacgcagaaggaaggccacagctgtacagaattgagaaagaatagagacctgcagttgaggccagcaggtcggctggactaactctccagccacagtaatgacccagacagagaaagccagactcataaagcttgctgagcaaaattaagggaacaaggttgagagccctagtaagcgaggctctaaaaagcacagctgagctgagatgggtgggcttctctgagtgcttctaaaatgcgctaaactgaggtgattactctgaggtaagcaaagctgggcttgagccaaaatgaagtagactgtaatgaactggaatgagctgggccgctaagctaaactaggctggcttaaccgagatgagccaaactggaatgaacttcattaatctaggttgaatagagctaaactctactgcctacactggactgttctgagctgagatgagctggggtgagctcagctatgctacgctgtgttggggtgagctgatctgaaatgagatactctggagtagctgagatggggtgagatggggtgagctgagctgggctgagctagactgagctgagctagggtgagctgagctgggtgagctgagctaagctggggtgagctgagctgagcttggctgagctagggtgagctgggctgagctggggtgagctgagctgagctggggtaagctgggatgagctggggtgagctgagctgagctggagtgagctgagctgggctgagctggggtgagctgggctgagctgggctgagctgggctgagctggggtgagctgagctggggtgagctgagctgagctggggtgagctgagctgagctggggtgagctggggtgagctgagctggggtgagctgagctgagctggggtgagctgagctggggtgagctgagctgagctggggtgagctgagctgagctgagctgagctgagctggggtgagctgagctgagctgagctggggtgagctggggtgagctgagctgagctggagtgagctgagctgggctgagctggggtgagctgggctgagctggggtgagctgagctgagctgagctgagctggggtgagctgagctgagctggggtgagctgagctggggtgagctgggctgagctgagctgagctgagctgagctgagctgagctgagctgagctgagctgagctgagctgagctgagctgagctgagctgagctggggtgagctgagctgagctgggctgagctggggtgagctgggctgagctgggctgagctgggctgagctggggtgagctgagctggggtgagctgagctgagctgggctgagctgagctgagctggggtgagctgagctgagctggggtgagctgagctgagctgagctggggtgagctgagctgagctgggctgagcagggctgagctggggtgagctgagctgagctggggtgagctgggctgagctgggctgagctgagctgagctgggctgagctgggctgagctgggctgagctgggctgagctgggctgagctggggtgagctgagctggggtgagctggggtgagctgagctggggtgagctgagctggggtgagctgagctgagctggggtgagctgagctggggtgagctgagctgagctggggtgagctgagctgagctggggtgagctgagctagggtgaactgggctgggtgagctggagtgagctgagctgaggtgaactggggtgagccgggatgttttgagttgagctggggtaagatgagctgaactggggtaaactgggatgagctgtggtgagcggagctggattgaactgagctgtgtgagctgagctggggtcagctgagcaagagtgagtagagctggctggccagaaccagaatcaattaggctaagtgagccagattgtgctgggatcagctgtactcagatgagctgggatgaggtaggctgggatgagctgggctagctgacatggattatgtgaggctgagctagcatgggctggcctagctgatgagctaagcttgaatgagcggggctgagctggactcagatgtgctagactgagctgtactggatgatctggtgtagggtgatctggactcaactgggctggctgatgggatgcgccaggttgaactaggctcagataagttaggctgagtagggcctggttgagatggttcgggatgagctgggaaaagatggactcggaccatgaactgggctgagctgggttgggagaccatgaattgagctgaactgagtgcagctgggataaactgggttgagctaagaatagactacctgaattgtgccaaactcggctgggatcaattggaaattatcaggatttagatgagccggactaaactatgctgagctggactggttggatgtgttgaactggcctgctgctgggctggcatagctgagttgaacttaaatgaggaaggctgagcaaggctagcctgcttgcatagagctgaactttagcctagcctgagctggaccagcctgagctgagtaggtctaaactgagttaaaaatcaacagggataatttaacagctaatttaacaagcctgaggtctgagattgaatgagcagagctgggatgaactgaatgagtttcaccaggcctggaccagttaggctaggacctcgttctatagaggcagactgtgtgctacagtggagtttcaagatgattccatgagtcctccccgcccccaacataacccaccttcctcctaccctacacgcctgtctggtgtgtaaatcccagctttgtgtgctgatacagaagcctgagcccctcccccacctccacctacctattactttgggatgagaatagttctcccagccagtgtctcagagggaagccaagcaggacaggcccaaggctacttgagaagccaggatctaggcctctccctgagaacgggtgttcatgcccctagagttggctgaagggccagatccacctactctagaggcatctctccctgtctgtgaaggcttccaaagtcacgttcctgtggctagaaggcagctccatagccctgctgcagtttcgtcctgtataccaggttcacctactaccatatctagccctgcctgccttaagagtagcaacaaggaaatagcagggtgtagagggatctcctgtctgacaggaggcaagaagacagattcttacccctccatttctcttttatccctctctggtcctcagagagtcagtccttcccaaatgtcttccccctcgtctcctgcgagagccccctgtctgataagaatctggtggccatgggctgcctggcccgggacttcctgcccagcaccatttccttcacctggaactaccagaacaacactgaagtcatccagggtatcagaaccttcccaacactgaggacagggggcaagtacctagccacctcgcaggtgttgctgtctcccaagagcatccttgaaggttcagatgaatacctggtatgcaaaatccactacggaggcaaaaacaaagatctgcatgtgcccattccaggtaagaaccaaaccctcccagcaggggtgcccaggcccaggcatggcccagagggagcagcggggtggggcttaggccaagctgagctcacaccttgacctttcattccagctgtcgcagagatgaaccccaatgtaaatgtgttcgtcccaccacgggatggcttctctggccctgcaccacgcaagtctaaactcatctgcgaggccacgaacttcactccaaaaccgatcacagtatcctggctaaaggatgggaagctcgtggaatctggcttcaccacagatccggtgaccatcgagaacaaaggatccacaccccaaacctacaaggtcataagcacacttaccatctctgaaatcgactggctgaacctgaatgtgtacacctgccgtgtggatcacaggggtctcaccttcttgaagaacgtgtcctccacatgtgctgccagtgagtggcctgggctaagcccaatgcctagccctcccagattagggaagtcctcctacaattatggccaatgccacccagacatggtcatttgctccttgaactttggctccccagagtggccaaggacaagaatgagcaataggcagtagaggggtgagaatcagctggaaggaccagcatcttcccttaagtaggtttgggggatggagactaagcttttttccaacttcacaactagatatgtcataacctgacacagtgttctcttgactgcaggtccctccacagacatcctaaccttcaccatccccccctcctttgccgacatcttcctcagcaagtccgctaacctgacctgtctggtctcaaacctggcaacctatgaaaccctgaatatctcctgggcttctcaaagtggtgaaccactggaaaccaaaattaaaatcatggaaagccctcccaatggcaccttcagtgctaagggtgtggctagtgtttgtgtggaagactggaataacaggaaggaatttgtgcgtactgtgactcacagggatctgccttcaccacagaagaaattcatctcaaaacccaatggtaggtatccccccttcccttcccctccaattgcaggacccttcctgtacctcatagggagggcaggtcctcttccaccctatcctcactactgtcttcatttacagaggtgcacaaacatccacctgctgtgtacctgctgccaccagctcgtgagcaactgaacctgagggagtcagccacagtcacctgcctggtgaagggcttctctcctgcagacatcagtgtgcagtggcttcagagagggcaactcttgccccaagagaagtatgtgaccagtgccccgatgccagagcctggggccccaggcttctactttacccacagcatcctgactgtgacagaggaggaatggaactccggagagacctatacctgtgttgtaggccacgaggccctgccacacctggtgaccgagaggaccgtggacaagtccactggtaaacccacactgtacaatgtctccctgatcatgtctgacacaggcggcacctgctattgaccatgctagcgctcaaccaggcaggccctgggtgtccagttgctctgtgtatgcaaactaaccatgtcagagtgagatgttgcattttataaaaattagaaataaaaaaaatccattcaaacgtcactggttttgattatacaatgctcatgcctgctgagacagttgtgttttgcttgctctgcacacaccctgcatacttgcctccaccctggcccttcctctaccttgccagtttcctccttgtgtgtgaactcagtcaggcttacaacagacagagtatgaacatgcgattcctccagctacttctagatatatggctgaaagcttgc

SEQ ID NO: 13 - protein, 4 aa, Artificial Sequence
  GLSG
GLSG

SEQ ID NO: 14 - protein, 6 aa, Artificial Sequence
  linker - GGGGS
GLSGSG

SEQ ID NO: 15 - protein, 8 aa, Artificial Sequence
  linker - GLSGLSGS
GLSGLSGS

SEQ ID NO: 16 - protein, 10 aa, Artificial Sequence
  GLSGLSGLSG linker
GLSGLSGLSG

SEQ ID NO: 17 - protein, 10 aa, Artificial Sequence
  GLSGGSGLSG
GLSGGSGLSG

SEQ ID NO: 18 - DNA, 20 bp, Artificial Sequence
  5' detect VH1-69 FR3
acagaagttccagggcagag

SEQ ID NO: 19 - DNA, 21 bp, Artificial Sequence
  3' up detect spec
tgtccactgggttcgtgcctt

SEQ ID NO: 20 - DNA, 21 bp, Artificial Sequence
  5' down detect spec
cagtatcagcccgtcatactt

SEQ ID NO: 21 - DNA, 19 bp, Artificial Sequence
  3' VH1-69 overlap detect
taacccctgtcatctcctc

SEQ ID NO: 22 - DNA, 23 bp, Artificial Sequence
  5' DNA Target(PAM)
ggatcctggtttagttaaagagg

SEQ ID NO: 23 - RNA, 42 nt, Artificial Sequence
  5' VH1-69 Cas9 crRNA
ggauccugguuuaguuaaagguuuuagagcuaugcuguuuug

SEQ ID NO: 24 - DNA, 23 bp, Artificial Sequence
  3' DNA Target(PAM)
gacaaaaaccctgagggagaagg

SEQ ID NO: 25 - RNA, 42 nt, Artificial Sequence
  3 VH1-69 Cas9 crRNA
gacaaaaacccugagggagaguuuuagagcuaugcuguuuug

SEQ ID NO: 26 - DNA, 19 bp, Artificial Sequence
  5' up detect VH1-69
ctgtgaaataccctgcctc

SEQ ID NO: 27 - DNA, 21 bp, Artificial Sequence
  3' up detect spec
tgtccactgggttcgtgcctt

SEQ ID NO: 28 - DNA, 21 bp, Artificial Sequence
  5' down detect spec
cagtatcagcccgtcatactt

SEQ ID NO: 29 - DNA, 20 bp, Artificial Sequence
  3'down detect M1116(h70)
ccccctcttgctctctttct

SEQ ID NO: 30 - DNA, 80 bp, Artificial Sequence
  VH1-69 MreI del Joiner Oligo
gtgaaaacccacatcctgagagtgacaaaaaccctgagggagaaggcagctgtgccgggctgaggagatgacaggggtta

SEQ ID NO: 31 - DNA, 20 bp, Artificial Sequence
  5' detect VH1-69 FR3
acagaagttccagggcagag

SEQ ID NO: 32 - DNA, 20 bp, Artificial Sequence
  3'down detect M1116(h70)
ccccctcttgctctctttct